European Patent Specification EP 3 512 606 B1, published July 19, 2023. Title: Nouvelle utilisation cosmétique et/ou nutraceutique ou dermatologique d'un extrait de levure. Applicant: BASF Beauty Care Solutions FR SAS. The sequence listing filed with the application follows.

SEQUENCE LISTING (6 sequences)

SEQ ID NO: 1 - DNA, 21 bp, artificial sequence
  amorce
tcagcagttgaagggacagat

SEQ ID NO: 2 - DNA, 22 bp, artificial sequence
  amorce
ccagaacaatgaatggttaagg

SEQ ID NO: 3 - DNA, 20 bp, artificial sequence
  amorce
ttacagagttaactgttacc

SEQ ID NO: 4 - DNA, 20 bp, artificial sequence
  amorce
atacaaatccagcacgctct

SEQ ID NO: 5 - DNA, 20 bp, artificial sequence
  amorce
agagtttgatcctggctcag

SEQ ID NO: 6 - DNA, 19 bp, artificial sequence
  amorce
tgctgcctcccgtaggagt